European Patent Application EP 4 342 979 A1, published March 27, 2024. Title: NOVEL METHOD. Applicant: BitBio Discovery. The sequence listing filed with the application follows.

SEQUENCE LISTING (25 sequences)

SEQ ID NO: 1 - DNA, 20 bp, synthetic construct
  source 1..20: mol_type = other DNA
gtcgagtcgcttctcgatta

SEQ ID NO: 2 - DNA, 21 bp, synthetic construct
  source 1..21: mol_type = other DNA
gtccctagtggccccactgtg

SEQ ID NO: 3 - DNA, 20 bp, synthetic construct
  source 1..20: mol_type = other DNA
cacgcgccacaccgtcgatc

SEQ ID NO: 4 - DNA, 21 bp, synthetic construct
  source 1..21: mol_type = other DNA
gttcgtctagaaagaaagact

SEQ ID NO: 5 - DNA, 20 bp, synthetic construct
  source 1..20: mol_type = other DNA
ggccaagggagggggaaagg

SEQ ID NO: 6 - DNA, 20 bp, synthetic construct
  source 1..20: mol_type = other DNA
ctgtccagtccccatttgag

SEQ ID NO: 7 - DNA, 20 bp, synthetic construct
  source 1..20: mol_type = other DNA
cagatggagcagtggatgac

SEQ ID NO: 8 - DNA, 20 bp, synthetic construct
  source 1..20: mol_type = other DNA
ctgtccagtccccatttgag

SEQ ID NO: 9 - DNA, 20 bp, synthetic construct
  source 1..20: mol_type = other DNA
cacgtcaccgcatgttagaa

SEQ ID NO: 10 - DNA, 22 bp, synthetic construct
  source 1..22: mol_type = other DNA
cgcggatatgagtctgtctaag

SEQ ID NO: 11 - DNA, 22 bp, synthetic construct
  source 1..22: mol_type = other DNA
agacactttacggctctgttgg

SEQ ID NO: 12 - DNA, 25 bp, synthetic construct
  source 1..25: mol_type = other DNA
tttcccatgattccttcatatttgc

SEQ ID NO: 13 - DNA, 24 bp, synthetic construct
  source 1..24: mol_type = other DNA
caaatcaaacatggctcagttgtg

SEQ ID NO: 14 - DNA, 20 bp, synthetic construct
  source 1..20: mol_type = other DNA
ccgcctccatccagtctatt

SEQ ID NO: 15 - DNA, 20 bp, synthetic construct
  source 1..20: mol_type = other DNA
gtgcacgagtgggttacatc

SEQ ID NO: 16 - DNA, 20 bp, synthetic construct
  source 1..20: mol_type = other DNA
gcgcgacgctaatccgtcga

SEQ ID NO: 17 - DNA, 20 bp, synthetic construct
  source 1..20: mol_type = other DNA
gtggtatataaggggtttta

SEQ ID NO: 18 - DNA, 20 bp, synthetic construct
  source 1..20: mol_type = other DNA
ggccaagggagggggaaagg

SEQ ID NO: 19 - DNA, 113 bp, synthetic construct
  source 1..113: mol_type = other DNA
  misc_feature 21..113: note = tcRNA sequence
  misc_feature 1..20: note = CRISPRa gRNA sequence
ggccaagggagggggaaagggtttcagagctatgctggaaacagcatagcaagttgaaataaggctagtccgttatcaacttgaaaaagtggcaccgagtcggtgcttttttt

SEQ ID NO: 20 - DNA, 265 bp, synthetic construct
  source 1..265: mol_type = other DNA
  misc_feature 1..20: note = CRISPRa gRNA sequence
  misc_feature 21..86: note = tcRNA sequence
  misc_feature 87..108: note = capture sequence 1
  misc_feature 109..132: note = tcRNA sequence
  misc_feature 133..152: note = Csy4 20nt recognition site
  misc_feature 153..172: note = CRISPRa gRNA sequence
  misc_feature 173..265: note = tcRNA sequence
gcgcgacgctaatccgtcgagtttaagagctaagctggaaacagcatagcaagtttaaataaggctagtccgttatcaacttggccgctttaaggccggtcctagcaaggccaagtggcaccgagtcggtgcgttcactgccgtataggcagggccaagggagggggaaagggtttcagagctatgctggaaacagcatagcaagttgaaataaggctagtccgttatcaacttgaaaaagtggcaccgagtcggtgcttttttt

SEQ ID NO: 21 - DNA, 265 bp, synthetic construct
  source 1..265: mol_type = other DNA
  misc_feature 1..20: note = CRISPRa gRNA sequence
  misc_feature 21..86: note = tcRNA sequence
  misc_feature 87..108: note = capture sequence 1
  misc_feature 109..132: note = tcRNA sequence
  misc_feature 133..152: note = Csy4 20nt recognition site
  misc_feature 153..172: note = CRISPRa gRNA sequence
  misc_feature 173..265: note = tcRNA sequence
gtggtatataaggggttttagtttaagagctaagctggaaacagcatagcaagtttaaataaggctagtccgttatcaacttggccgctttaaggccggtcctagcaaggccaagtggcaccgagtcggtgcgttcactgccgtataggcagggccaagggagggggaaagggtttcagagctatgctggaaacagcatagcaagttgaaataaggctagtccgttatcaacttgaaaaagtggcaccgagtcggtgcttttttt

SEQ ID NO: 22 - DNA, 19 bp, synthetic construct
  source 1..19: mol_type = other DNA
tccctatcagtgatagaga

SEQ ID NO: 23 - DNA, 4194 bp, synthetic construct
  source 1..4194: mol_type = other DNA
  misc_feature 1..823: note = 5-prime CLYBL gene homology arm
  misc_feature 836..862: note = splice acceptor sequence
  misc_feature 863..886: note = linker
  misc_feature 887..940: note = T2A sequence
  misc_feature 950..1549: note = puromycin resistance gene
  polyA_site 1587..1811: note = bGH polyA sequence
  misc_feature 1822..2371: note = insulator sequence
  regulatory 2372..2611: note = hU6 promoter; regulatory_class = promoter
  misc_feature 2612..2631: note = CRISPRa gRNA sequence
  misc_feature 2632..2724: note = tcRNA sequence
  misc_feature 2737..3296: note = insulator sequence
  misc_feature 3319..4194: note = 3-prime CLYBL gene homology arm
gaactctgccacctaatttaggatcccagactctcctactggagacacaggtccttagtgacagtctgcaccaccattcagacaagtcagtagggccatcttagatcatccagccctagtcaagccaccagataactgtacccacataagtgacccctggcgagacgagcaggagaatcatgccaatgggccaatatacattctgacccacagtttcataataaaataaaatggttgtggttgtaagccactatgtttcagagtggtttgttacacagcaataaataactaatatagtaggcataccatcaagtccaaagtaggtagagaagaatgtaaatagcagagcaaaacagcatgactggtggctgggaggcttaaaactgggacaggatcagagtcatgaaagaagtcaaagaaatggttcagaagtaaggctgagactgacttacaaaagctgaaagtccctttaagttggtgtttggtgcattggcaggggcaggtatggtgacttaaaagagccatgctcaacaagatcaagcacaacacaatcacgggtcaccccagcagaccttagcgagtctagccatttctttggtggtggtcacagtcatgcttcagcccagtttccacttggacaaatggtacatattttcaatgagatgaaaattaagatacaatccatgtgctcagagagtgatcacagctctgactaaacactgtgccccaaagtgttgaggaattgggaaaacctagctgagttagtgatctcttttctgttacaataaagctcataatgaaaattagccttctttgttcttccggtacggcaagcttctgacctcttctcttcctcccacagggcctcgagagatctggcagcggagagggcagaggaagtcttctaacatgcggtgacgtggaggagaatcccggccctaggctcgagatgaccgagtacaagcccacggtgcgcctcgccacccgcgacgacgtccccagggccgtacgcaccctcgccgccgcgttcgccgactaccccgccacgcgccacaccgtcgatccggaccgccacatcgagcgggtcaccgagctgcaagaactcttcctcacgcgcgtcgggctcgacatcggcaaggtgtgggtcgcggacgacggcgccgcggtggcggtctggaccacgccggagagcgtcgaagcgggggcggtgttcgccgagatcggcccgcgcatggccgagttgagcggttcccggctggccgcgcagcaacagatggaaggcctcctggcgccgcaccggcccaaggagcccgcgtggttcctggccaccgtcggcgtctcgcccgaccaccagggcaagggtctgggcagcgccgtcgtgctccccggagtggaggcggccgagcgcgccggggtgcccgccttcctggagacctccgcgccccgcaacctccccttctacgagcggctcggcttcaccgtcaccgccgacgtcgaggtgcccgaaggaccgcgcacctggtgcatgacccgcaagcccggtgcctgatctagagggcccgtttaaacccgctgatcagcctcgactgtgccttctagttgccagccatctgttgtttgcccctcccccgtgccttccttgaccctggaaggtgccactcccactgtcctttcctaataaaatgaggaaattgcatcgcattgtctgagtaggtgtcattctattctggggggtggggtggggcaggacagcaagggggaggattgggaagacaatagcaggcatgctggggatgcggtgggctctatggtcactcgagttagacagactcatatccgcgggagctcacggggacagccccccccccaaagcccccagggctgtaattgcgttcctctcccgctagggggcggcagcgagccgcccagggctccgctccggcccgacgctccccccgcatccccgagccggagcccgcagcgtgcggggacagcccggcacggggaaggtggcacgggatcgctttcctctgaacgcttctcgctgctctttgagcctgcagacacctggggggatacggggaaaaagctttatctagatccgcgggagctcacggggacagcccccccccaaagcccccagggctgtaattgcgttcctctcccgctagggggcagcagcgagccgcccggggctccgctccggcccgacgctccccccgcatccccgagccggagcccgcagcgtgcggggacagcccggcacggggaaggtggcacgggatcgctttcctctgaacgcttctcactgctctttgagcctgcagacacctggggggatacggggaaaaagctttatcgctctgtcgcatttcccatgattccttcatatttgcatatacgatacaaggctgttagagagataattagaattaatttgactgtaaacacaaagatattagtacaaaatacgtgacgtagaaagtaataatttcttgggtagtttgcagttttaaaattatgttttaaaatggactatcatatgcttaccgtaacttgaaagtatttcgatttcttggctttatatatcttgtggaaaggacgaaacaccggccaagggagggggaaagggtttcagagctatgctggaaacagcatagcaagttgaaataaggctagtccgttatcaacttgaaaaagtggcaccgagtcggtgctttttttcttgacagtactcctactggcggacagagcgataaagctttttccccgtatccccccaggtgtctgcaggctcaaagagcagtgagaagcgttcagaggaaagcgatcccgtgccaccttccccgtgccgggctgtccccgcacgctgcgggctccggctcggggatgcggggggagcgtcgggccggagcggagccccgggcggctcgctgctgccccctagcgggagaggaacgcaattacagccctgggggctttgggggggggctgtccccgtgagctcccgcggatctagataaagctttttccccgtatccccccaggtgtctgcaggctcaaagagcagcgagaagcgttcagaggaaagcgatcccgtgccaccttccccgtgccgggctgtccccgcacgctgcgggctccggctcggggatgcggggggagcgtcgggccggagcggagccccgggcggctcgctgctgccccctagcgggagaggaacgcaattacagccctgggggctttgggggggggctgtccccgtgagctcccgcggatatgagtctgtctaagtgcttaagtcgacttactcgactttcagactgttatttcttgacttttaaatgtaagatattatctactgacttccttctatgtaagatgaggattgagctctcttacccttctcccatttcctcatccttccaacataaatatattttgggattatatcaacattcaatgttacttaaagtgaccttgtaaatattttcacaactgagccatgtttgatttgtatacttatgtttactttactgtttttcctgaagttaataattgccttgaatttatttatttctttaaaaatgtttcattactcaggactgtagtttacattacgattctttgtgttatacagttgatgggtttcttttctttcttaatttctttaaaaaatagagatggggtcttactatattacccaggctggtcttgaagtcctgggctcaagtgatcttcctgtctcagcctaccaagtagctgagactataggtgcaaaaaagccactatacctggctagtttacaggttttaacaaatgcattatgccacgtatccattattacaggatcacacaagatattttcattaccctgaaagcatccctgtgttccaccaattcatcctgcctccatgagccgctggcaaccactgatctctatagttttgccttttctaaaatgtcatataattggaatcatacagtctgtagcattttcagactagcttttaaaatttggcaatatgcatttaaggttcctccttaaatgtgaagggcatagccaatgtggcttgatagctcatttctttttattggtgaatatttcattgtctggatgttccacagtttgtttatccattcacctattcaatttgctttttttctgtgtatctatcactaattcaatactgg

SEQ ID NO: 24 - DNA, 9150 bp, synthetic construct
  source 1..9150: mol_type = other DNA
  misc_feature 1..801: note = 5-prime AAVS1 gene homology arm
  misc_feature 809..835: note = splice acceptor sequence
  misc_feature 836..859: note = linker
  misc_feature 860..913: note = T2A sequence
  misc_feature 923..1522: note = puromycin resistance gene
  polyA_site 1560..1784: note = bGH polyA sequence
  regulatory 1791..2140: note = TRE3G promoter; regulatory_class = promoter
  misc_feature 2166..2186: note = nuclear localisation sequence
  misc_feature 2187..2210: note = linker
  misc_feature 2211..6347: note = dCas9 sequence
  misc_feature 6348..6359: note = linker
  misc_feature 6360..6383: note = nuclear localisation sequence
  misc_feature 6384..8027: note = VPR sequence
  polyA_site 8207..8288: note = SV40 polyA sequence
  misc_feature 8316..9150: note = 3-prime AAVS1 gene homology arm
tgctttctctgaccagcattctctcccctgggcctgtgccgctttctgtctgtagcttgtggcctgggtcacctctacggctggcccagatccttccctgccgcctccttcaggttccgtcttcctccactccctcttccccttgctctctgctgtgttgctgcccaaggatgctctttccggagcacttccttctcggcgctgcaccacgtgatgtcctctgagcggatcctccccgtgtctgggtcctctccgggcatctctcctccctcacccaaccccatgccgtcttcactcgctgggttcccttttccttctccttctggggcctgtgccatctctcgtttcttaggatggccttctccgacggatgtctcccttgcgtcccgcctccccttcttgtaggcctgcatcatcaccgtttttctggacaaccccaaagtaccccgtctccctggctttagccacctctccatcctcttgctttctttgcctggacaccccgttctcctgtggattcgggtcacctctcactcctttcatttgggcagctcccctaccccccttacctctctagtctgtgctagctcttccagccccctgtcatggcatcttccaggggtccgagagctcagctagtcttcttcctccaacccgggcccctatgtccacttcaggacagcatgtttgctgcctccagggatcctgtgtccccgagctgggaccaccttatattcccagggccggttaatgtggctctggttctgggtacttttatctgtcccctccaccccacagtggggcaagcttctgacctcttctcttcctcccacagggcctcgagagatctggcagcggagagggcagaggaagtcttctaacatgcggtgacgtggaggagaatcccggccctaggctcgagatgaccgagtacaagcccacggtgcgcctcgccacccgcgacgacgtccccagggccgtacgcaccctcgccgccgcgttcgccgactaccccgccacgcgccacaccgtcgatccggaccgccacatcgagcgggtcaccgagctgcaagaactcttcctcacgcgcgtcgggctcgacatcggcaaggtgtgggtcgcggacgacggcgccgcggtggcggtctggaccacgccggagagcgtcgaagcgggggcggtgttcgccgagatcggcccgcgcatggccgagttgagcggttcccggctggccgcgcagcaacagatggaaggcctcctggcgccgcaccggcccaaggagcccgcgtggttcctggccaccgtcggcgtctcgcccgaccaccagggcaagggtctgggcagcgccgtcgtgctccccggagtggaggcggccgagcgcgccggggtgcccgccttcctggagacctccgcgccccgcaacctccccttctacgagcggctcggcttcaccgtcaccgccgacgtcgaggtgcccgaaggaccgcgcacctggtgcatgacccgcaagcccggtgcctgatctagagggcccgtttaaacccgctgatcagcctcgactgtgccttctagttgccagccatctgttgtttgcccctcccccgtgccttccttgaccctggaaggtgccactcccactgtcctttcctaataaaatgaggaaattgcatcgcattgtctgagtaggtgtcattctattctggggggtggggtggggcaggacagcaagggggaggattgggaagacaatagcaggcatgctggggatgcggtgggctctatggtcactcgagtttactccctatcagtgatagagaacgtatgaagagtttactccctatcagtgatagagaacgtatgcagactttactccctatcagtgatagagaacgtataaggagtttactccctatcagtgatagagaacgtatgaccagtttactccctatcagtgatagagaacgtatctacagtttactccctatcagtgatagagaacgtatatccagtttactccctatcagtgatagagaacgtatgtcgaggtaggcgtgtacggtgggcgcctataaaagcagagctcgtttagtgaaccgtcagatcgcctggagcaattccacaacacttttgtcttatacttagtagaaggagaggccaccatggccccaaagaagaagcggaaggtcggtatccacggagtcccagcagccgacaagaagtacagcatcggcctggccatcggcaccaactctgtgggctgggccgtgatcaccgacgagtacaaggtgcccagcaagaaattcaaggtgctgggcaacaccgaccggcacagcatcaagaagaacctgatcggcgccctgctgttcgacagcggagaaacagccgaggccacccggctgaagagaaccgccagaagaagatacaccagacggaagaaccggatctgctatctgcaagagatcttcagcaacgagatggccaaggtggacgacagcttcttccacagactggaagagtccttcctggtggaagaggataagaagcacgagcggcaccccatcttcggcaacatcgtggacgaggtggcctaccacgagaagtaccccaccatctaccacctgagaaagaaactggtggacagcaccgacaaggccgacctgcggctgatctatctggccctggcccacatgatcaagttccggggccacttcctgatcgagggcgacctgaaccccgacaacagcgacgtggacaagctgttcatccagctggtgcagacctacaaccagctgttcgaggaaaaccccatcaacgccagcggcgtggacgccaaggccatcctgtctgccagactgagcaagagcagacggctggaaaatctgatcgcccagctgcccggcgagaagaagaatggcctgttcggcaacctgattgccctgagcctgggcctgacccccaacttcaagagcaacttcgacctggccgaggatgccaaactgcagctgagcaaggacacctacgacgacgacctggacaacctgctggcccagatcggcgaccagtacgccgacctgtttctggccgccaagaacctgtccgacgccatcctgctgagcgacatcctgagagtgaacaccgagatcaccaaggcccccctgagcgcctctatgatcaagagatacgacgagcaccaccaggacctgaccctgctgaaagctctcgtgcggcagcagctgcctgagaagtacaaagagattttcttcgaccagagcaagaacggctacgccggctacatcgatggcggagccagccaggaagagttctacaagttcatcaagcccatcctggaaaagatggacggcaccgaggaactgctcgtgaagctgaacagagaggacctgctgcggaagcagcggaccttcgacaacggcagcatcccccaccagatccacctgggagagctgcacgccattctgcggcggcaggaagatttttacccattcctgaaggacaaccgggaaaagatcgagaagatcctgaccttccgcatcccctactacgtgggccctctggccaggggaaacagcagattcgcctggatgaccagaaagagcgaggaaaccatcaccccctggaacttcgaggaagtggtggacaagggcgccagcgcccagagcttcatcgagcggatgaccaacttcgataagaacctgcccaacgagaaggtgctgcccaagcacagcctgctgtacgagtacttcaccgtgtacaacgagctgaccaaagtgaaatacgtgaccgagggaatgagaaagcccgccttcctgagcggcgagcagaaaaaagccatcgtggacctgctgttcaagaccaaccggaaagtgaccgtgaagcagctgaaagaggactacttcaagaaaatcgagtgcttcgactccgtggaaatctccggcgtggaagatcggttcaacgcctccctgggcacataccacgatctgctgaaaattatcaaggacaaggacttcctggacaatgaggaaaacgaggacattctggaagatatcgtgctgaccctgacactgtttgaggacagagagatgatcgaggaacggctgaaaacctatgcccacctgttcgacgacaaagtgatgaagcagctgaagcggcggagatacaccggctggggcaggctgagccggaagctgatcaacggcatccgggacaagcagtccggcaagacaatcctggatttcctgaagtccgacggcttcgccaacagaaacttcatgcagctgatccacgacgacagcctgacctttaaagaggacatccagaaagcccaggtgtccggccagggcgatagcctgcacgagcacattgccaatctggccggcagccccgccattaagaagggcatcctgcagacagtgaaggtggtggacgagctcgtgaaagtgatgggccggcacaagcccgagaacatcgtgatcgaaatggccagagagaaccagaccacccagaagggacagaagaacagccgcgagagaatgaagcggatcgaagagggcatcaaagagctgggcagccagatcctgaaagaacaccccgtggaaaacacccagctgcagaacgagaagctgtacctgtactacctgcagaatgggcgggatatgtacgtggaccaggaactggacatcaaccggctgtccgactacgatgtggacgctatcgtgcctcagagctttctgaaggacgactccatcgataacaaagtgctgactcggagcgacaagaaccggggcaagagcgacaacgtgccctccgaagaggtcgtgaagaagatgaagaactactggcgccagctgctgaatgccaagctgattacccagaggaagttcgacaatctgaccaaggccgagagaggcggcctgagcgaactggataaggccggcttcatcaagagacagctggtggaaacccggcagatcacaaagcacgtggcacagatcctggactcccggatgaacactaagtacgacgagaacgacaaactgatccgggaagtgaaagtgatcaccctgaagtccaagctggtgtccgatttccggaaggatttccagttttacaaagtgcgcgagatcaacaactaccaccacgcccacgacgcctacctgaacgccgtcgtgggaaccgccctgatcaaaaagtaccctaagctggaaagcgagttcgtgtacggcgactacaaggtgtacgacgtgcggaagatgatcgccaagagcgagcaggaaatcggcaaggctaccgccaagtacttcttctacagcaacatcatgaactttttcaagaccgagattaccctggccaacggcgagatccggaagcggcctctgatcgagacaaacggcgaaacaggcgagatcgtgtgggataagggccgggactttgccaccgtgcggaaagtgctgtctatgccccaagtgaatatcgtgaaaaagaccgaggtgcagacaggcggcttcagcaaagagtctatcctgcccaagaggaacagcgacaagctgatcgccagaaagaaggactgggaccctaagaagtacggcggcttcgacagccccaccgtggcctattctgtgctggtggtggccaaagtggaaaagggcaagtccaagaaactgaagagtgtgaaagagctgctggggatcaccatcatggaaagaagcagcttcgagaagaatcccatcgactttctggaagccaagggctacaaagaagtgaaaaaggacctgatcatcaagctgcctaagtactccctgttcgagctggaaaacggccggaagagaatgctggcctctgccggcgaactgcagaagggaaacgaactggccctgccctccaaatatgtgaacttcctgtacctggccagccactatgagaagctgaagggctcccccgaggataatgagcagaaacagctgtttgtggaacagcacaaacactacctggacgagatcatcgagcagatcagcgagttctccaagagagtgatcctggccgacgctaatctggacaaggtgctgagcgcctacaacaagcacagagacaagcctatcagagagcaggccgagaatatcatccacctgtttaccctgaccaatctgggagcccctgccgccttcaagtactttgacaccaccatcgaccggaagaggtacaccagcaccaaagaggtgctggacgccaccctgatccaccagagcatcaccggcctgtacgagacacggatcgacctgtctcagctgggaggcgacgcctatccctatgacgtgcccgattatgccagcctgggcagcggctcccccaagaaaaaacgcaaggtggaaagcggctctgagactcccggcacatccgaaagcgcaacccctgagtctgaggccagcggttccggacgggctgacgcattggacgattttgatctggatatgctgggaagtgacgccctcgatgattttgaccttgacatgcttggttcggatgcccttgatgactttgacctcgacatgctcggcagtgacgcccttgatgatttcgacctggacatgctgattaactctagaagttccggatctccgaaaaagaaacgcaaagttggtagccagtacctgcccgacaccgacgaccggcaccggatcgaggaaaagcggaagcggacctacgagacattcaagagcatcatgaagaagtcccccttcagcggccccaccgaccctagacctccacctagaagaatcgccgtgcccagcagatccagcgccagcgtgccaaaacctgccccccagccttaccccttcaccagcagcctgagcaccatcaactacgacgagttccctaccatggtgttccccagcggccagatctctcaggcctctgctctggctccagcccctcctcaggtgctgcctcaggctcctgctcctgcaccagctccagccatggtgtctgcactggctcaggcaccagcacccgtgcctgtgctggctcctggacctccacaggctgtggctccaccagcccctaaacctacacaggccggcgagggcacactgtctgaagctctgctgcagctgcagttcgacgacgaggatctgggagccctgctgggaaacagcaccgatcctgccgtgttcaccgacctggccagcgtggacaacagcgagttccagcagctgctgaaccagggcatccctgtggcccctcacaccaccgagcccatgctgatggaataccccgaggccatcacccggctcgtgacaggcgctcagaggcctcctgatccagctcctgcccctctgggagcaccaggcctgcctaatggactgctgtctggcgacgaggacttcagctctatcgccgatatggatttctcagccttgctgggctctggcagcggcagccgggattccagggaagggatgtttttgccgaagcctgaggccggctccgctattagtgacgtgtttgagggccgcgaggtgtgccagccaaaacgaatccggccatttcatcctccaggaagtccatgggccaaccgcccactccccgccagcctcgcaccaacaccaaccggtccagtacatgagccagtcgggtcactgaccccggcaccagtccctcagccactggatccagcgcccgcagtgactcccgaggccagtcacctgttggaggatcccgatgaagagacgagccaggctgtcaaagcccttcgggagatggccgatactgtgattccccagaaggaagaggctgcaatctgtggccaaatggacctttcccatccgcccccaaggggccatctggatgagctgacaaccacacttgagtccatgaccgaggatctgaacctggactcacccctgaccccggaattgaacgagattctggataccttcctgaacgacgagtgcctcttgcatgccatgcatatcagcacaggactgtccatcttcgacacatctctgttttaaccggggatcctctagtcagctgacgcgtgctagcgcggccgcatcgataagcttgtcgacgatatctctagaggatcataatcagccataccacatttgtagaggttttacttgctttaaaaaacctcccacacctccccctgaacctgaaacataaaatgaatgcaattgttgttgttaacttgtttattgcagcttataatggttacaaataaagcaatagcatcacaaatttcacaaataaagcatttttttcactgccttgacagtactcttaagtcgacttactagggacaggattggtgacagaaaagccccatccttaggcctcctccttcctagtctcctgatattgggtctaacccccacctcctgttaggcagattccttatctggtgacacacccccatttcctggagccatctctctccttgccagaacctctaaggtttgcttacgatggagccagagaggatcctgggagggagagcttggcagggggtgggagggaagggggggatgcgtgacctgcccggttctcagtggccaccctgcgctaccctctcccagaacctgagctgctctgacgcggctgtctggtgcgtttcactgatcctggtgctgcagcttccttacacttcccaagaggagaagcagtttggaaaaacaaaatcagaataagttggtcctgagttctaactttggctcttcacctttctagtccccaatttatattgttcctccgtgcgtcagttttacctgtgagataaggccagtagccagccccgtcctggcagggctgtggtgaggaggggggtgtccgtgtggaaaactccctttgtgagaatggtgcgtcctaggtgttcaccaggtcgtggccgcctctactccctttctctttctccatccttctttccttaaagagtccccagtgctatctgggacatattcctccgcccagagcagggtcccgcttccctaaggccctgctctgggcttctgggtttgagtccttggcaagcccaggagaggcgctcaggcttccctgtcccccttcctcgtccaccatctcatgcccctggctctcctgccccttccctacaggggttcctggctctgctct

SEQ ID NO: 25 - DNA, 9771 bp, synthetic construct
  source 1..9771: mol_type = other DNA
  misc_feature 1..801: note = 5-prime AAVS1 gene homology arm
  misc_feature 809..835: note = splice acceptor sequence
  misc_feature 836..859: note = linker
  misc_feature 860..913: note = nuclear localisation sequence
  misc_feature 923..1522: note = puromycin resistance gene
  polyA_site 1560..1784: note = bGH polyA sequence
  regulatory 1791..2140: note = TRE3G promoter; regulatory_class = promoter
  misc_feature 2161..2725: note = Csy4 sequence
  misc_feature 2726..2779: note = T2A sequence
  misc_feature 2780..2786: note = linker
  misc_feature 2787..2807: note = nuclear localisation sequence
  misc_feature 2808..2831: note = linker
  misc_feature 2832..6968: note = dCas9 sequence
  misc_feature 6981..7004: note = linker
  misc_feature 7005..8648: note = VPR sequence
  polyA_site 8828..8909: note = SV40 polyA sequence
  misc_feature 8937..9771: note = 3-prime AAVS1 gene homology arm
tgctttctctgaccagcattctctcccctgggcctgtgccgctttctgtctgtagcttgtggcctgggtcacctctacggctggcccagatccttccctgccgcctccttcaggttccgtcttcctccactccctcttccccttgctctctgctgtgttgctgcccaaggatgctctttccggagcacttccttctcggcgctgcaccacgtgatgtcctctgagcggatcctccccgtgtctgggtcctctccgggcatctctcctccctcacccaaccccatgccgtcttcactcgctgggttcccttttccttctccttctggggcctgtgccatctctcgtttcttaggatggccttctccgacggatgtctcccttgcgtcccgcctccccttcttgtaggcctgcatcatcaccgtttttctggacaaccccaaagtaccccgtctccctggctttagccacctctccatcctcttgctttctttgcctggacaccccgttctcctgtggattcgggtcacctctcactcctttcatttgggcagctcccctaccccccttacctctctagtctgtgctagctcttccagccccctgtcatggcatcttccaggggtccgagagctcagctagtcttcttcctccaacccgggcccctatgtccacttcaggacagcatgtttgctgcctccagggatcctgtgtccccgagctgggaccaccttatattcccagggccggttaatgtggctctggttctgggtacttttatctgtcccctccaccccacagtggggcaagcttctgacctcttctcttcctcccacagggcctcgagagatctggcagcggagagggcagaggaagtcttctaacatgcggtgacgtggaggagaatcccggccctaggctcgagatgaccgagtacaagcccacggtgcgcctcgccacccgcgacgacgtccccagggccgtacgcaccctcgccgccgcgttcgccgactaccccgccacgcgccacaccgtcgatccggaccgccacatcgagcgggtcaccgagctgcaagaactcttcctcacgcgcgtcgggctcgacatcggcaaggtgtgggtcgcggacgacggcgccgcggtggcggtctggaccacgccggagagcgtcgaagcgggggcggtgttcgccgagatcggcccgcgcatggccgagttgagcggttcccggctggccgcgcagcaacagatggaaggcctcctggcgccgcaccggcccaaggagcccgcgtggttcctggccaccgtcggcgtctcgcccgaccaccagggcaagggtctgggcagcgccgtcgtgctccccggagtggaggcggccgagcgcgccggggtgcccgccttcctggagacctccgcgccccgcaacctccccttctacgagcggctcggcttcaccgtcaccgccgacgtcgaggtgcccgaaggaccgcgcacctggtgcatgacccgcaagcccggtgcctgatctagagggcccgtttaaacccgctgatcagcctcgactgtgccttctagttgccagccatctgttgtttgcccctcccccgtgccttccttgaccctggaaggtgccactcccactgtcctttcctaataaaatgaggaaattgcatcgcattgtctgagtaggtgtcattctattctggggggtggggtggggcaggacagcaagggggaggattgggaagacaatagcaggcatgctggggatgcggtgggctctatggtcactcgagtttactccctatcagtgatagagaacgtatgaagagtttactccctatcagtgatagagaacgtatgcagactttactccctatcagtgatagagaacgtataaggagtttactccctatcagtgatagagaacgtatgaccagtttactccctatcagtgatagagaacgtatctacagtttactccctatcagtgatagagaacgtatatccagtttactccctatcagtgatagagaacgtatgtcgaggtaggcgtgtacggtgggcgcctataaaagcagagctcgtttagtgaaccgtcagatcgcctggagcaattccacaacacttttgtcttatacttagtagaaggagaggccaccaatgggtgaccactatctcgacatcagattgcgaccggatcccgagttccctcctgcgcaactgatgtccgtactgtttgggaaattgcaccaagccctcgtcgcgcaaggcggcgataggataggcgttagttttcctgatctcgatgagtcaagatcccgactcggtgagcgcctgcgaatacatgcttcagcagatgacctcagggcacttctggctcggccgtggttggagggtcttagggaccatttgcaatttggtgaacccgccgtcgtcccgcatccaaccccatatcggcaagtaagcagagtccaggctaaatcaaaccccgagagattgaggcggcggcttatgcgacgccacgatctctccgaggaagaggctcgaaaacggataccggacacggtggccagggcactcgacctgccatttgtaacccttcgctcccagtccactggtcaacatttccgattgtttattagacacggtcctttgcaggtgactgctgaggaggggggatttacatgctacggactcagcaaagggggttttgtcccgtggttttgagggcagaggaagtctgttaacatgcggtgacgtcgaggagaatcctggcccaatgggccccaaagaagaagcggaaggtcggtatccacggagtcccagcagccgacaagaagtacagcatcggcctggccatcggcaccaactctgtgggctgggccgtgatcaccgacgagtacaaggtgcccagcaagaaattcaaggtgctgggcaacaccgaccggcacagcatcaagaagaacctgatcggcgccctgctgttcgacagcggagaaacagccgaggccacccggctgaagagaaccgccagaagaagatacaccagacggaagaaccggatctgctatctgcaagagatcttcagcaacgagatggccaaggtggacgacagcttcttccacagactggaagagtccttcctggtggaagaggataagaagcacgagcggcaccccatcttcggcaacatcgtggacgaggtggcctaccacgagaagtaccccaccatctaccacctgagaaagaaactggtggacagcaccgacaaggccgacctgcggctgatctatctggccctggcccacatgatcaagttccggggccacttcctgatcgagggcgacctgaaccccgacaacagcgacgtggacaagctgttcatccagctggtgcagacctacaaccagctgttcgaggaaaaccccatcaacgccagcggcgtggacgccaaggccatcctgtctgccagactgagcaagagcagacggctggaaaatctgatcgcccagctgcccggcgagaagaagaatggcctgttcggcaacctgattgccctgagcctgggcctgacccccaacttcaagagcaacttcgacctggccgaggatgccaaactgcagctgagcaaggacacctacgacgacgacctggacaacctgctggcccagatcggcgaccagtacgccgacctgtttctggccgccaagaacctgtccgacgccatcctgctgagcgacatcctgagagtgaacaccgagatcaccaaggcccccctgagcgcctctatgatcaagagatacgacgagcaccaccaggacctgaccctgctgaaagctctcgtgcggcagcagctgcctgagaagtacaaagagattttcttcgaccagagcaagaacggctacgccggctacatcgatggcggagccagccaggaagagttctacaagttcatcaagcccatcctggaaaagatggacggcaccgaggaactgctcgtgaagctgaacagagaggacctgctgcggaagcagcggaccttcgacaacggcagcatcccccaccagatccacctgggagagctgcacgccattctgcggcggcaggaagatttttacccattcctgaaggacaaccgggaaaagatcgagaagatcctgaccttccgcatcccctactacgtgggccctctggccaggggaaacagcagattcgcctggatgaccagaaagagcgaggaaaccatcaccccctggaacttcgaggaagtggtggacaagggcgccagcgcccagagcttcatcgagcggatgaccaacttcgataagaacctgcccaacgagaaggtgctgcccaagcacagcctgctgtacgagtacttcaccgtgtacaacgagctgaccaaagtgaaatacgtgaccgagggaatgagaaagcccgccttcctgagcggcgagcagaaaaaagccatcgtggacctgctgttcaagaccaaccggaaagtgaccgtgaagcagctgaaagaggactacttcaagaaaatcgagtgcttcgactccgtggaaatctccggcgtggaagatcggttcaacgcctccctgggcacataccacgatctgctgaaaattatcaaggacaaggacttcctggacaatgaggaaaacgaggacattctggaagatatcgtgctgaccctgacactgtttgaggacagagagatgatcgaggaacggctgaaaacctatgcccacctgttcgacgacaaagtgatgaagcagctgaagcggcggagatacaccggctggggcaggctgagccggaagctgatcaacggcatccgggacaagcagtccggcaagacaatcctggatttcctgaagtccgacggcttcgccaacagaaacttcatgcagctgatccacgacgacagcctgacctttaaagaggacatccagaaagcccaggtgtccggccagggcgatagcctgcacgagcacattgccaatctggccggcagccccgccattaagaagggcatcctgcagacagtgaaggtggtggacgagctcgtgaaagtgatgggccggcacaagcccgagaacatcgtgatcgaaatggccagagagaaccagaccacccagaagggacagaagaacagccgcgagagaatgaagcggatcgaagagggcatcaaagagctgggcagccagatcctgaaagaacaccccgtggaaaacacccagctgcagaacgagaagctgtacctgtactacctgcagaatgggcgggatatgtacgtggaccaggaactggacatcaaccggctgtccgactacgatgtggacgctatcgtgcctcagagctttctgaaggacgactccatcgataacaaagtgctgactcggagcgacaagaaccggggcaagagcgacaacgtgccctccgaagaggtcgtgaagaagatgaagaactactggcgccagctgctgaatgccaagctgattacccagaggaagttcgacaatctgaccaaggccgagagaggcggcctgagcgaactggataaggccggcttcatcaagagacagctggtggaaacccggcagatcacaaagcacgtggcacagatcctggactcccggatgaacactaagtacgacgagaacgacaaactgatccgggaagtgaaagtgatcaccctgaagtccaagctggtgtccgatttccggaaggatttccagttttacaaagtgcgcgagatcaacaactaccaccacgcccacgacgcctacctgaacgccgtcgtgggaaccgccctgatcaaaaagtaccctaagctggaaagcgagttcgtgtacggcgactacaaggtgtacgacgtgcggaagatgatcgccaagagcgagcaggaaatcggcaaggctaccgccaagtacttcttctacagcaacatcatgaactttttcaagaccgagattaccctggccaacggcgagatccggaagcggcctctgatcgagacaaacggcgaaacaggcgagatcgtgtgggataagggccgggactttgccaccgtgcggaaagtgctgtctatgccccaagtgaatatcgtgaaaaagaccgaggtgcagacaggcggcttcagcaaagagtctatcctgcccaagaggaacagcgacaagctgatcgccagaaagaaggactgggaccctaagaagtacggcggcttcgacagccccaccgtggcctattctgtgctggtggtggccaaagtggaaaagggcaagtccaagaaactgaagagtgtgaaagagctgctggggatcaccatcatggaaagaagcagcttcgagaagaatcccatcgactttctggaagccaagggctacaaagaagtgaaaaaggacctgatcatcaagctgcctaagtactccctgttcgagctggaaaacggccggaagagaatgctggcctctgccggcgaactgcagaagggaaacgaactggccctgccctccaaatatgtgaacttcctgtacctggccagccactatgagaagctgaagggctcccccgaggataatgagcagaaacagctgtttgtggaacagcacaaacactacctggacgagatcatcgagcagatcagcgagttctccaagagagtgatcctggccgacgctaatctggacaaggtgctgagcgcctacaacaagcacagagacaagcctatcagagagcaggccgagaatatcatccacctgtttaccctgaccaatctgggagcccctgccgccttcaagtactttgacaccaccatcgaccggaagaggtacaccagcaccaaagaggtgctggacgccaccctgatccaccagagcatcaccggcctgtacgagacacggatcgacctgtctcagctgggaggcgacgcctatccctatgacgtgcccgattatgccagcctgggcagcggctcccccaagaaaaaacgcaaggtggaaagcggctctgagactcccggcacatccgaaagcgcaacccctgagtctgaggccagcggttccggacgggctgacgcattggacgattttgatctggatatgctgggaagtgacgccctcgatgattttgaccttgacatgcttggttcggatgcccttgatgactttgacctcgacatgctcggcagtgacgcccttgatgatttcgacctggacatgctgattaactctagaagttccggatctccgaaaaagaaacgcaaagttggtagccagtacctgcccgacaccgacgaccggcaccggatcgaggaaaagcggaagcggacctacgagacattcaagagcatcatgaagaagtcccccttcagcggccccaccgaccctagacctccacctagaagaatcgccgtgcccagcagatccagcgccagcgtgccaaaacctgccccccagccttaccccttcaccagcagcctgagcaccatcaactacgacgagttccctaccatggtgttccccagcggccagatctctcaggcctctgctctggctccagcccctcctcaggtgctgcctcaggctcctgctcctgcaccagctccagccatggtgtctgcactggctcaggcaccagcacccgtgcctgtgctggctcctggacctccacaggctgtggctccaccagcccctaaacctacacaggccggcgagggcacactgtctgaagctctgctgcagctgcagttcgacgacgaggatctgggagccctgctgggaaacagcaccgatcctgccgtgttcaccgacctggccagcgtggacaacagcgagttccagcagctgctgaaccagggcatccctgtggcccctcacaccaccgagcccatgctgatggaataccccgaggccatcacccggctcgtgacaggcgctcagaggcctcctgatccagctcctgcccctctgggagcaccaggcctgcctaatggactgctgtctggcgacgaggacttcagctctatcgccgatatggatttctcagccttgctgggctctggcagcggcagccgggattccagggaagggatgtttttgccgaagcctgaggccggctccgctattagtgacgtgtttgagggccgcgaggtgtgccagccaaaacgaatccggccatttcatcctccaggaagtccatgggccaaccgcccactccccgccagcctcgcaccaacaccaaccggtccagtacatgagccagtcgggtcactgaccccggcaccagtccctcagccactggatccagcgcccgcagtgactcccgaggccagtcacctgttggaggatcccgatgaagagacgagccaggctgtcaaagcccttcgggagatggccgatactgtgattccccagaaggaagaggctgcaatctgtggccaaatggacctttcccatccgcccccaaggggccatctggatgagctgacaaccacacttgagtccatgaccgaggatctgaacctggactcacccctgaccccggaattgaacgagattctggataccttcctgaacgacgagtgcctcttgcatgccatgcatatcagcacaggactgtccatcttcgacacatctctgttttaaccggggatcctctagtcagctgacgcgtgctagcgcggccgcatcgataagcttgtcgacgatatctctagaggatcataatcagccataccacatttgtagaggttttacttgctttaaaaaacctcccacacctccccctgaacctgaaacataaaatgaatgcaattgttgttgttaacttgtttattgcagcttataatggttacaaataaagcaatagcatcacaaatttcacaaataaagcatttttttcactgccttgacagtactcttaagtcgacttactagggacaggattggtgacagaaaagccccatccttaggcctcctccttcctagtctcctgatattgggtctaacccccacctcctgttaggcagattccttatctggtgacacacccccatttcctggagccatctctctccttgccagaacctctaaggtttgcttacgatggagccagagaggatcctgggagggagagcttggcagggggtgggagggaagggggggatgcgtgacctgcccggttctcagtggccaccctgcgctaccctctcccagaacctgagctgctctgacgcggctgtctggtgcgtttcactgatcctggtgctgcagcttccttacacttcccaagaggagaagcagtttggaaaaacaaaatcagaataagttggtcctgagttctaactttggctcttcacctttctagtccccaatttatattgttcctccgtgcgtcagttttacctgtgagataaggccagtagccagccccgtcctggcagggctgtggtgaggaggggggtgtccgtgtggaaaactccctttgtgagaatggtgcgtcctaggtgttcaccaggtcgtggccgcctctactccctttctctttctccatccttctttccttaaagagtccccagtgctatctgggacatattcctccgcccagagcagggtcccgcttccctaaggccctgctctgggcttctgggtttgagtccttggcaagcccaggagaggcgctcaggcttccctgtcccccttcctcgtccaccatctcatgcccctggctctcctgccccttccctacaggggttcctggctctgctct